European Patent Specification EP 4 322 983 B1, published June 24, 2026. Title: Treatment of cerebrovascular events and neurological disorders. Applicant: UNIVERSITY COLLEGE CORK NATIONAL UNIVERSITY OF IRELAND CORK. The sequence listing filed with the application follows.

SEQUENCE LISTING (3 sequences)

SEQ ID NO: 1 - protein, 419 aa, Homo sapiens
MGTLSAPPCTQRIKWKGLLLTASLLNFWNLPTTAQVTIEAEPTKVSEGKDVLLLVHNLPQNLTGYIWYKGQMRDLYHYITSYVVDGEIIIYGPAYSGRETAYSNASLLIQNVTREDAGSYTLHIIKGDDGTRGVTGRFTFTLHLETPKPSISSSNLNPRETMEAVSLTCDPETPDASYLWWMNGQSLPMTHSLKLSETNRTLFLLGVTKYTAGPYECEIRNPVSASRSDPVTLNLLPKLPKPYITINNLNPRENKDVLNFTCEPKSENYTYIWWLNGQSLPVSPRVKRPIENRILILPSVTRNETGPYQCEIRDRYGGIRSDPVTLNVLYGPDLPRIYPSFTYYRSGEVLYLSCSADSNPPAQYSWTINEKFQLPGQKLFIRHITTKHSGLYVCSVRNSATGKESSKSMTVEVSDWTVP

SEQ ID NO: 2 - DNA, 1956 bp, Artificial Sequence
  PSG1-Fc ORF
atgggaaccctctcagcccctccctgcacacagcgcatcaaatggaaggggctcctgctcacagcatcacttttaaacttctggaacctgcccaccactgcccaagtcacgattgaagccgagccaaccaaagtttccgaggggaaggatgttcttctacttgtccacaatttgccccagaatcttaccggctacatctggtacaaagggcaaatgagggacctctaccattacattacatcatatgtagtagacggtgaaataattatatatgggcctgcatatagtggacgagaaacagcatattccaatgcatccctgctgatccagaatgtcacccgggaggacgcaggatcctacaccttacacatcataaagggagatgatgggactagaggagtaactggacgtttcaccttcaccttacacctggagactcctaagccctccatctccagcagcaacttaaatcccagggagaccatggaggctgtgagcttaacctgtgaccctgagactccagacgcaagctacctgtggtggatgaatggtcagagcctccctatgactcacagcttgaagctgtccgaaaccaacaggaccctctttctattgggtgtcacaaagtatactgcaggaccctatgaatgtgaaatacggaacccagtgagtgccagccgcagtgacccagtcaccctgaatctcctcccgaagctgcccaagccctacatcaccatcaacaacttaaaccccagggagaataaggatgtcttaaacttcacctgtgaacctaagagtgagaactacacctacatttggtggctaaatggtcagagcctcccggtcagtcccagggtaaagcgacccattgaaaacaggatcctcattctacccagtgtcacgagaaatgaaacaggaccctatcaatgtgaaatacgggaccgatatggtggcatccgcagtgacccagtcaccctgaatgtcctctatggtccagacctccccagaatttacccttcattcacctattaccgttcaggagaagtcctctacttgtcctgttctgcggactctaacccaccggcacagtattcttggacaattaatgaaaagtttcagctaccaggacaaaagctctttatccgccatattactacaaagcatagcgggctctatgtttgctctgttcgtaactcagccactggcaaggaaagctccaaatccatgacagtcgaagtctctgactggacagttcccgagcccaaatcttgtgacaaaactcacacatgcccaccgtgcccagcacctgaactcctggggggaccgtcagtcttcctcttccccccaaaacccaaggacaccctctacatcacccgggaacctgaggtcacatgcgtggtggtggacgtgagccacgaagaccctgaggtcaagttcaactggtacgtggacggcgtggaggtgcataatgccaagacaaagccgcgggaggagcagtacaacagcacgtaccgtgtggtcagcgtcctcaccgtcctgcaccaggactggctgaatggcaaggagtacaagtgcaaggtctccaacaaagccctcccagcccccatcgagaaaaccatctccaaagccaaagggcagccccgagaaccacaggtgtacaccctgcccccatcccgggatgagctgaccaagaaccaggtcagcctgacctgcctggtcaaaggcttctatcccagcgacatcgccgtggagtgggagagcaatgggcagccggagaacaactacaagaccacgcctcccgtgctggactccgacggctccttcttcctctacagcaagctcaccgtggacaagagcaggtggcagcaggggaacgtcttctcatgctccgtgatgcatgaggctctgaagttccactacacgcagaagagcctctccctgtctccgggtaaatga

SEQ ID NO: 3 - DNA, 699 bp, Artificial Sequence
  Modified human Fc ORF
gagcccaaatcttgtgacaaaactcacacatgcccaccgtgcccagcacctgaactcctggggggaccgtcagtcttcctcttccccccaaaacccaaggacaccctctacatcacccgggaacctgaggtcacatgcgtggtggtggacgtgagccacgaagaccctgaggtcaagttcaactggtacgtggacggcgtggaggtgcataatgccaagacaaagccgcgggaggagcagtacaacagcacgtaccgtgtggtcagcgtcctcaccgtcctgcaccaggactggctgaatggcaaggagtacaagtgcaaggtctccaacaaagccctcccagcccccatcgagaaaaccatctccaaagccaaagggcagccccgagaaccacaggtgtacaccctgcccccatcccgggatgagctgaccaagaaccaggtcagcctgacctgcctggtcaaaggcttctatcccagcgacatcgccgtggagtgggagagcaatgggcagccggagaacaactacaagaccacgcctcccgtgctggactccgacggctccttcttcctctacagcaagctcaccgtggacaagagcaggtggcagcaggggaacgtcttctcatgctccgtgatgcatgaggctctgaagttccactacacgcagaagagcctctccctgtctccgggtaaatga